European Patent Application EP 4 137 518 A1, published February 22, 2023. Title: NON-PLATELET DEPLETING AND NON-RED BLOOD CELL DEPLETING CD47 ANTIBODIES AND METHODS OF USE THEREOF. Applicant: Inhibrx, Inc. The sequence listing filed with the application follows.

SEQUENCE LISTING (147 sequences)

SEQ ID NO: 1 - protein, 330 aa, Homo sapiens [sequence omitted]

SEQ ID NO: 2 - protein, 326 aa, Homo sapiens
ASTKGPSVFPLAPCSRSTSESTAALGCLVKDYFPEPVTVSWNSGALTSGVHTFPAVLQSSGLYSLSSVVTVPSSNFGTQTYTCNVDHKPSNTKVDKTVERKCCVECPPCPAPPVAGPSVFLFPPKPKDTLMISRTPEVTCVVVDVSHEDPEVQFNWYVDGVEVHNAKTKPREEQFNSTFRVVSVLTVVHQDWLNGKEYKCKVSNKGLPAPIEKTISKTKGQPREPQVYTLPPSREEMTKNQVSLTCLVKGFYPSDISVEWESNGQPENNYKTTPPMLDSDGSFFLYSKLTVDKSRWQQGNVFSCSVMHEALHNHYTQKSLSLSPGK

SEQ ID NO: 3 - protein, 377 aa, Homo sapiens
ASTKGPSVFPLAPCSRSTSGGTAALGCLVKDYFPEPVTVSWNSGALTSGVHTFPAVLQSSGLYSLSSVVTVPSSSLGTQTYTCNVNHKPSNTKVDKRVELKTPLGDTTHTCPRCPEPKSCDTPPPCPRCPEPKSCDTPPPCPRCPEPKSCDTPPPCPRCPAPELLGGPSVFLFPPKPKDTLMISRTPEVTCVVVDVSHEDPEVQFKWYVDGVEVHNAKTKPREEQYNSTFRVVSVLTVLHQDWLNGKEYKCKVSNKALPAPIEKTISKTKGQPREPQVYTLPPSREEMTKNQVSLTCLVKGFYPSDIAVEWESSGQPENNYNTTPPMLDSDGSFFLYSKLTVDKSRWQQGNIFSCSVMHEALHNRFTQKSLSLSPGK

SEQ ID NO: 4 - protein, 327 aa, Homo sapiens
ASTKGPSVFPLAPCSRSTSESTAALGCLVKDYFPEPVTVSWNSGALTSGVHTFPAVLQSSGLYSLSSVVTVPSSSLGTKTYTCNVDHKPSNTKVDKRVESKYGPPCPSCPAPEFLGGPSVFLFPPKPKDTLMISRTPEVTCVVVDVSQEDPEVQFNWYVDGVEVHNAKTKPREEQFNSTYRVVSVLTVLHQDWLNGKEYKCKVSNKGLPSSIEKTISKAKGQPREPQVYTLPPSQEEMTKNQVSLTCLVKGFYPSDIAVEWESNGQPENNYKTTPPVLDSDGSFFLYSRLTVDKSRWQEGNVFSCSVMHEALHNHYTQKSLSLSLGK

SEQ ID NO: 5 - protein, 118 aa, synthetic construct
  REGION 1..118: note = Variable heavy chain region of a humanized CD47 antibody
EVQLQQSGAELVRSGASVKLSCTASGFNIKDYYLHWVKQRPEQGLEWIGWIDPDNGDTEFAPKFQGKATMTADTSSNTAYLQLSSLTSEDTAVYYCNAAYGSSSYPMDYWGQGTSVTV

SEQ ID NO: 6 - protein, 118 aa, synthetic construct
  REGION 1..118: note = Variable heavy chain region of a humanized CD47 antibody
EVQLVQSGAEVKKPGATVKISCKVSGFNIKDYYLHWVQQAPGKGLEWMGWIDPDNGDTEYAEKFQGRVTITADTSTDTAYMELSSLRSEDTAVYYCNAAYGSSSYPMDYWGQGTTVTV

SEQ ID NO: 7 - protein, 118 aa, synthetic construct
  REGION 1..118: note = Variable heavy chain region of a humanized CD47 antibody
QMQLVQSGAEVKKTGSSVKVSCKASGFNIKDYYLHWVRQAPGQALEWMGWIDPDNGDTEYAQKFQDRVTITRDRSMSTAYMELSSLRSEDTAMYYCNAAYGSSSYPMDYWGQGTTVTV

SEQ ID NO: 8 - protein, 118 aa, synthetic construct
  REGION 1..118: note = Variable heavy chain region of a humanized CD47 antibody
EVQLVQSGAEVKKTGSSVKVSCKASGFNIKDYYLHWVRQAPGQALEWMGWIDPDNGDTEYAQKFQDRVTITRDRSMSTAYMELSSLRSEDTAMYYCNAAYGSSSYPMDYWGQGTTVTV

SEQ ID NO: 9 - protein, 118 aa, synthetic construct
  REGION 1..118: note = Variable heavy chain region of a humanized CD47 antibody
QMQLVQSGAEVKKTGSSVKVSCKASGFNIKDYYLHWVRQAPGQALEWMGWIDPDNGDTEYAQKFQGRVTMTADTSSNTAYMELSSLRSEDTAMYYCNAAYGSSSYPMDYWGQGTTVTV

SEQ ID NO: 10 - protein, 118 aa, synthetic construct
  REGION 1..118: note = Variable heavy chain region of a humanized CD47 antibody
QMQLVQSGAEVKKTGSSVKVSCKASGFNIKDYYLHWVRQAPGQALEWMGWIDPDNGDTEYAQKFQGRVTMTEDTSTDTAYMELSSLRSEDTAMYYCNAAYGSSSYPMDYWGQGTTVTV

SEQ ID NO: 11 - protein, 118 aa, synthetic construct
  REGION 1..118: note = Variable heavy chain region of a humanized CD47 antibody
QMQLVQSGAEVKKTGSSVKVSCKASGFNIKDYYLHWVRQAPGQALEWMGWIDPDQGDTEYAQKFQDRVTITRDRSMSTAYMELSSLRSEDTAMYYCNAAYGSSSYPMDYWGQGTTVTV

SEQ ID NO: 12 - protein, 118 aa, synthetic construct
  REGION 1..118: note = Variable heavy chain region of a humanized CD47 antibody
QMQLVQSGAEVKKTGSSVKVSCKASGFNIKDYYLHWVRQAPGQALEWMGWIDPDYGDTEYAQKFQDRVTITRDRSMSTAYMELSSLRSEDTAMYYCNAAYGSSSYPMDYWGQGTTVTV

SEQ ID NO: 13 - protein, 118 aa, synthetic construct
  REGION 1..118: note = Variable heavy chain region of a humanized CD47 antibody
QMQLVQSGAEVKKTGSSVKVSCKASGFNIKDYYLHWVRQAPGQALEWMGWIDPDSGDTEYAQKFQDRVTITRDRSMSTAYMELSSLRSEDTAMYYCNAAYGSSSYPMDYWGQGTTVTV

SEQ ID NO: 14 - protein, 118 aa, synthetic construct
  REGION 1..118: note = Variable heavy chain region of a humanized CD47 antibody
QMQLVQSGAEVKKTGSSVKVSCKASGFNIKDYYLHWVRQAPGQALEWMGWIDPDNADTEYAQKFQDRVTITRDRSMSTAYMELSSLRSEDTAMYYCNAAYGSSSYPMDYWGQGTTVTV

SEQ ID NO: 15 - protein, 118 aa, synthetic construct
  REGION 1..118: note = Variable heavy chain region of a humanized CD47 antibody
QMQLVQSGAEVKKTGSSVKVSCKASGFNIKDYYLHWVRQAPGQALEWMGWIDPDNTDTEYAQKFQDRVTITRDRSMSTAYMELSSLRSEDTAMYYCNAAYGSSSYPMDYWGQGTTVTV

SEQ ID NO: 16 - protein, 118 aa, synthetic construct
  REGION 1..118: note = Variable heavy chain region of a humanized CD47 antibody
QMQLVQSGAEVKKTGSSVKVSCKASGFNIKDYYLHWVRQAPGQALEWMGWIDPDNGDTEYAQKFQDRVTITRDRSMSTAYMELSSLRSEDTAMYYCNAAYGSSPYPMDYWGQGTTVTV

SEQ ID NO: 17 - protein, 118 aa, synthetic construct
  REGION 1..118: note = Variable heavy chain region of a humanized CD47 antibody
QMQLVQSGAEVKKTGSSVKVSCKASGYTFTYYYLHWVRQAPGQALEWMGWIDPDNGDTEYAQKFQDRVTITRDRSMSTAYMELSSLRSEDTAMYYCNAAYGSSSYPMDYWGQGTTVTV

SEQ ID NO: 18 - protein, 118 aa, synthetic construct
  REGION 1..118: note = Variable heavy chain region of a humanized CD47 antibody
QMQLVQSGAEVKKTGSSVKVSCKASGFTFTYYYLHWVRQAPGQALEWMGWIDPDNGDTEYAQKFQDRVTITRDRSMSTAYMELSSLRSEDTAMYYCNAAYGSSSYPMDYWGQGTTVTV

SEQ ID NO: 19 - protein, 118 aa, synthetic construct
  REGION 1..118: note = Variable heavy chain region of a humanized CD47 antibody
QMQLVQSGAEVKKTGSSVKVSCKASGYNFTYYYLHWVRQAPGQALEWMGWIDPDNGDTEYAQKFQDRVTITRDRSMSTAYMELSSLRSEDTAMYYCNAAYGSSSYPMDYWGQGTTVTV

SEQ ID NO: 20 - protein, 118 aa, synthetic construct
  REGION 1..118: note = Variable heavy chain region of a humanized CD47 antibody
QMQLVQSGAEVKKTGSSVKVSCKASGYTITYYYLHWVRQAPGQALEWMGWIDPDNGDTEYAQKFQDRVTITRDRSMSTAYMELSSLRSEDTAMYYCNAAYGSSSYPMDYWGQGTTVTV

SEQ ID NO: 21 - protein, 118 aa, synthetic construct
  REGION 1..118: note = Variable heavy chain region of a humanized CD47 antibody
QMQLVQSGAEVKKTGSSVKVSCKASGYTFKYYYLHWVRQAPGQALEWMGWIDPDNGDTEYAQKFQDRVTITRDRSMSTAYMELSSLRSEDTAMYYCNAAYGSSSYPMDYWGQGTTVTV

SEQ ID NO: 22 - protein, 118 aa, synthetic construct
  REGION 1..118: note = Variable heavy chain region of a humanized CD47 antibody
QMQLVQSGAEVKKTGSSVKVSCKASGYTFTDYYLHWVRQAPGQALEWMGWIDPDNGDTEYAQKFQDRVTITRDRSMSTAYMELSSLRSEDTAMYYCNAAYGSSSYPMDYWGQGTTVTV

SEQ ID NO: 23 - protein, 118 aa, synthetic construct
  REGION 1..118: note = Variable heavy chain region of a humanized CD47 antibody
QMQLVQSGAEVKKTGSSVKVSCKASGFTFTDYYLHWVRQAPGQALEWMGWIDPDNGDTEYAQKFQDRVTITRDRSMSTAYMELSSLRSEDTAMYYCNAAYGSSSYPMDYWGQGTTVTV

SEQ ID NO: 24 - protein, 118 aa, synthetic construct
  REGION 1..118: note = Variable heavy chain region of a humanized CD47 antibody
QMQLVQSGAEVKKTGSSVKVSCKASGFTITDYYLHWVRQAPGQALEWMGWIDPDNGDTEYAQKFQDRVTITRDRSMSTAYMELSSLRSEDTAMYYCNAAYGSSSYPMDYWGQGTTVTV

SEQ ID NO: 25 - protein, 118 aa, synthetic construct
  REGION 1..118: note = Variable heavy chain region of a humanized CD47 antibody
QMQLVQSGAEVKKTGSSVKVSCKASGYTFKDYYLHWVRQAPGQALEWMGWIDPDNGDTEYAQKFQDRVTITRDRSMSTAYMELSSLRSEDTAMYYCNAAYGSSSYPMDYWGQGTTVTV

SEQ ID NO: 26 - protein, 118 aa, synthetic construct
  REGION 1..118: note = Variable heavy chain region of a humanized CD47 antibody
QMQLVQSGAEVKKTGSSVKVSCKASGFTFKDYYLHWVRQAPGQALEWMGWIDPDNGDTEYAQKFQDRVTITRDRSMSTAYMELSSLRSEDTAMYYCNAAYGSSSYPMDYWGQGTTVTV

SEQ ID NO: 27 - protein, 118 aa, synthetic construct
  REGION 1..118: note = Variable heavy chain region of a humanized CD47 antibody
QMQLVQSGAEVKKTGSSVKVSCKASGFNIKDYYLHWVRQAPGQALEWMGWIDPDNGDTEYAQKFQDRVTITRDRSMSTAYLQLSSLRSEDTAMYYCNAAYGSSSYPMDYWGQGTTVTV

SEQ ID NO: 28 - protein, 118 aa, synthetic construct
  REGION 1..118: note = Variable heavy chain region of a humanized CD47 antibody
QMQLVQSGAEVKKTGSSVKVSCKASGFNIKDYYLHWVRQAPGQALEWMGWIDPDNGDTEYAQKFQDRVTITRDRSMSTAYMELSSLTSEDTAVYYCNAAYGSSSYPMDYWGQGTTVTV

SEQ ID NO: 29 - protein, 118 aa, synthetic construct
  REGION 1..118: note = Variable heavy chain region of a humanized CD47 antibody
EVQLVQSGAEVKKPGATVKISCKVSGFNIKDYYLHWVRQAPGQALEWMGWIDPDNGDTEYAQKFQDRVTITRDRSMSTAYMELSSLRSEDTAMYYCNAAYGSSSYPMDYWGQGTTVTV

SEQ ID NO: 30 - protein, 118 aa, synthetic construct
  REGION 1..118: note = Variable heavy chain region of a humanized CD47 antibody
EVQLVQSGAEVKKPGATVKISCKVSGFNIKDYYLHWVQQAPGKGLEWMGWIDPDNGDTEYAQKFQDRVTITRDRSMSTAYMELSSLRSEDTAMYYCNAAYGSSSYPMDYWGQGTTVTV

SEQ ID NO: 31 - protein, 107 aa, synthetic construct
  REGION 1..107: note = Variable light chain region of a humanized CD47 antibody
DIKMTQSPSSLYASLGERVTITCKASQDIHRYLSWFQQKPGKSPKILIYRANRLVDGVPSRFSGSGSGQDYSLTISSLEYEDMGIYYCLQYDEFPYTFGGGTKLEMK

SEQ ID NO: 32 - protein, 107 aa, synthetic construct
  REGION 1..107: note = Variable light chain region of a humanized CD47 antibody
DIKMTQSPSSLYASLGERVTITCKASQDIHRYLSWFQQKPGKSPKILIYRANRLVDGVPSRFSGSGSGQDYSLTISSLEYEDMGIYYCLQYDEFPYTFGGGTKLEIK

SEQ ID NO: 33 - protein, 107 aa, synthetic construct
  REGION 1..107: note = Variable light chain region of a humanized CD47 antibody
DIQMTQSPSSLSASVGDRVTITCKASQDIHRYLSWYQQKPGKAPKLLIYRANRLVDGVPSRFSGSGSGTDFTFTISSLQPEDIATYYCLQYDEFPYTFGGGTKVEIK

SEQ ID NO: 34 - protein, 107 aa, synthetic construct
  REGION 1..107: note = Variable light chain region of a humanized CD47 antibody
DIQMTQSPSSLSASVGDRVTITCKASQDIHRYLSWFQQKPGKAPKSLIYRANRLVDGVPSRFSGSGSGTDFTLTISSLQPEDFATYYCLQYDEFPYTFGGGTKVEIK

SEQ ID NO: 35 - protein, 107 aa, synthetic construct
  REGION 1..107: note = Variable light chain region of a humanized CD47 antibody
NIQMTQSPSAMSASVGDRVTITCKASQDIHRYLSWFQQKPGKVPKHLIYRANRLVDGVPSRFSGSGSGTEFTLTISSLQPEDFATYYCLQYDEFPYTFGGGTKVEIK

SEQ ID NO: 36 - protein, 107 aa, synthetic construct
  REGION 1..107: note = Variable light chain region of a humanized CD47 antibody
DIQMTQSPSSLSASVGDRVTITCKASQDIHRYLSWYQQKPGKAPKRLIYRANRLVDGVPSRFSGSGSGTEFTLTISSLQPEDFATYYCLQYDEFPYTFGGGTKVEIK

SEQ ID NO: 37 - protein, 107 aa, synthetic construct
  REGION 1..107: note = Variable light chain region of a humanized CD47 antibody
DIQMTQSPSSLSASVGDRVTITCRASQDIHRYLAWYQQKPGKVPKLLIYRANRLQSGVPSRFSGSGSGTDFTLTISSLQPEDVATYYCLQYDEFPYTFGQGTKVEIK

SEQ ID NO: 38 - protein, 107 aa, synthetic construct
  REGION 1..107: note = Variable light chain region of a humanized CD47 antibody
EIVLTQSPATLSLSPGERATLSCRASQDIHRYLAWYQQKPGQAPRLLIYRANRRATGIPARFSGSGSGTDFTLTISSLEPEDFAVYYCLQYDEFPYTGFQGTRLEIK

SEQ ID NO: 39 - protein, 107 aa, synthetic construct
  REGION 1..107: note = Variable light chain region of a humanized CD47 antibody
DIQMTQSPSAMSASVGDRVTITCKASQDIHRYLSWFQQKPGKVPKHLIYRANRLVDGVPSRFSGSGSGTEFTLTISSLQPEDFATYYCLQYDEFPYTFGGGTKVEIK

SEQ ID NO: 40 - protein, 107 aa, synthetic construct
  REGION 1..107: note = Variable light chain region of a humanized CD47 antibody
NIQMTQSPSAMSASVGDRVTITCRARQGIHRYLSWFQQKPGKVPKHLIYRANRLVDGVPSRFSGSGSGTEFTLTISSLQPEDFATYYCLQYDEFPYTFGGGTKVEIK

SEQ ID NO: 41 - protein, 107 aa, synthetic construct
  REGION 1..107: note = Variable light chain region of a humanized CD47 antibody
NIQMTQSPSAMSASVGDRVTITCKASQDIHRYLSWFQQKPGKVPKILIYRANRLVDGVPSRFSGSGSGTEFTLTISSLQPEDFATYYCLQYDEFPYTFGGGTKVEIK

SEQ ID NO: 42 - protein, 107 aa, synthetic construct
  REGION 1..107: note = Variable light chain region of a humanized CD47 antibody
NIQMTQSPSAMSASVGDRVTITCKASQDIHRYLSWFQQKPGKVPKHLIYRANRLVSGVPSRFSGSGSGTEFTLTISSLQPEDFATYYCLQYDEFPYTFGGGTKVEIK

SEQ ID NO: 43 - protein, 107 aa, synthetic construct
  REGION 1..107: note = Variable light chain region of a humanized CD47 antibody
NIQMTQSPSAMSASVGDRVTITCRARQGIHRYLSWFQQKPGKVPKILIYRANRLVDGVPSRFSGSGSGTEFTLTISSLQPEDFATYYCLQYDEFPYTFGGGTKVEIK

SEQ ID NO: 44 - protein, 107 aa, synthetic construct
  REGION 1..107: note = Variable light chain region of a humanized CD47 antibody
NIQMTQSPSAMSASVGDRVTITCRARQGIHRYLSWFQQKPGKVPKHLIYRANRLVSGVPSRFSGSGSGTEFTLTISSLQPEDFATYYCLQYDEFPYTFGGGTKVEIK

SEQ ID NO: 45 - protein, 107 aa, synthetic construct
  REGION 1..107: note = Variable light chain region of a humanized CD47 antibody
NIQMTQSPSAMSASVGDRVTITCKASQDIHRYLSWFQQKPGKVPKLLIYRANRLVDGVPSRFSGSGSGTEFTLTISSLQPEDFATYYCLQYDEFPYTFGGGTKVEIK

SEQ ID NO: 46 - protein, 107 aa, synthetic construct
  REGION 1..107: note = Variable light chain region of a humanized CD47 antibody
NIQMTQSPSAMSASVGDRVTITCKASQDIHRYLSWFQQKPGKVPKLLIYRANRLVSGVPSRFSGSGSGTEFTLTISSLQPEDFATYYCLQYDEFPYTFGGGTKVEIK

SEQ ID NO: 47 - protein, 107 aa, synthetic construct
  REGION 1..107: note = Variable light chain region of a humanized CD47 antibody
NIQMTQSPSAMSASVGDRVTITCRARQGIHRYLSWFQQKPGKVPKLLIYRANRLVSGVPSRFSGSGSGTEFTLTISSLQPEDFATYYCLQYDEFPYTFGGGTKVEIK

SEQ ID NO: 48 - protein, 323 aa, Homo sapiens
MWPLVAALLLGSACCGSAQLLFNKTKSVEFTFCNDTVVIPCFVTNMEAQNTTEVYVKWKFKGRDIYTFDGALNKSTVPTDFSSAKIEVSQLLKGDASLKMDKSDAVSHTGNYTCEVTELTREGETIIELKYRVVSWFSPNENILIVIFPIFAILLFWGQFGIKTLKYRSGGMDEKTIALLVAGLVITVIVIVGAILFVPGEYSLKNATGLGLIVTSTGILILLHYYVFSTAIGLTSFVIAILVIQVIAYILAVVGLSLCIAACIPMHGPLLISGLSILALAQLLGLVYMKFVASNQKTIQPPRKAVEEPLNAFKESKGMMNDE

SEQ ID NO: 49 - protein, 116 aa, Homo sapiens
QLLFNKTKSVEFTFCNDTVVIPCFVTNMEAQNTTEVYVKWKFKGRDIYTFDGALNKSTVPTDFSSAKIEVSQLLKGDASLKMDKSDAVSHTGNYTCEVTELTREGETIIELKYRVV

SEQ ID NO: 50 - protein, 10 aa, synthetic construct
  REGION 1..10: note = amino acid sequence of VH CDR1
GFNIKDYYLH

SEQ ID NO: 51 - protein, 10 aa, synthetic construct
  REGION 1..10: note = amino acid sequence of VH CDR2
WIDPDNGDTE

SEQ ID NO: 52 - protein, 13 aa, synthetic construct
  REGION 1..13: note = amino acid sequence of VH CDR3
NAAYGSSSYPMDY

SEQ ID NO: 53 - protein, 11 aa, synthetic construct
  REGION 1..11: note = amino acid sequence of VL CDR1
KASQDIHRYLS

SEQ ID NO: 54 - protein, 7 aa, synthetic construct
  REGION 1..7: note = amino acid sequence of VL CDR2
RANRLVD

SEQ ID NO: 55 - protein, 9 aa, synthetic construct
  REGION 1..9: note = amino acid sequence of VL CDR3
LQYDEFPYT

SEQ ID NO: 56 - protein, 4 aa, Homo sapiens
KGRD

SEQ ID NO: 57 - protein, 10 aa, synthetic construct
  REGION 1..10: note = amino acid sequence of VH CDR1
GYTFTYYYLH

SEQ ID NO: 58 - protein, 10 aa, synthetic construct
  REGION 1..10: note = amino acid sequence of VH CDR1
GFTFTYYYLH

SEQ ID NO: 59 - protein, 10 aa, synthetic construct
  REGION 1..10: note = amino acid sequence of VH CDR1
GYNFTYYYLH

SEQ ID NO: 60 - protein, 10 aa, synthetic construct
  REGION 1..10: note = amino acid sequence of VH CDR1
GYTITYYYLH

SEQ ID NO: 61 - protein, 10 aa, synthetic construct
  REGION 1..10: note = amino acid sequence of VH CDR1
GYTFKYYYLH

SEQ ID NO: 62 - protein, 10 aa, synthetic construct
  REGION 1..10: note = amino acid sequence of VH CDR1
GYTFTDYYLH

SEQ ID NO: 63 - protein, 10 aa, synthetic construct
  REGION 1..10: note = amino acid sequence of VH CDR1
GFTFTDYYLH

SEQ ID NO: 64 - protein, 10 aa, synthetic construct
  REGION 1..10: note = amino acid sequence of VH CDR1
GFTITDYYLH

SEQ ID NO: 65 - protein, 10 aa, synthetic construct
  REGION 1..10: note = amino acid sequence of VH CDR1
GYTFKDYYLH

SEQ ID NO: 66 - protein, 10 aa, synthetic construct
  REGION 1..10: note = amino acid sequence of VH CDR1
GFTFKDYYLH

SEQ ID NO: 67 - protein, 11 aa, synthetic construct
  REGION 1..11: note = amino acid sequence of VL CDR1
RASQDIHRYLA

SEQ ID NO: 68 - protein, 11 aa, synthetic construct
  REGION 1..11: note = amino acid sequence of VL CDR1
RARQGIHRYLS

SEQ ID NO: 69 - protein, 7 aa, synthetic construct
  REGION 1..7: note = amino acid sequence of VL CDR2
RANRLQS

SEQ ID NO: 70 - protein, 7 aa, synthetic construct
  REGION 1..7: note = amino acid sequence of VL CDR2
RANRRAT

SEQ ID NO: 71 - protein, 7 aa, synthetic construct
  REGION 1..7: note = amino acid sequence of VL CDR2
RANRLVS

SEQ ID NO: 72 - protein, 10 aa, synthetic construct
  REGION 1..10: note = amino acid sequence of VH CDR1
WIDPDQGDTE

SEQ ID NO: 73 - protein, 10 aa, synthetic construct
  REGION 1..10: note = amino acid sequence of VH CDR1
WIDPDYGDTE

SEQ ID NO: 74 - protein, 10 aa, synthetic construct
  REGION 1..10: note = amino acid sequence of VH CDR1
WIDPDSGDTE

SEQ ID NO: 75 - protein, 10 aa, synthetic construct
  REGION 1..10: note = amino acid sequence of VH CDR1
WIDPDNADTE

SEQ ID NO: 76 - protein, 10 aa, synthetic construct
  REGION 1..10: note = amino acid sequence of VH CDR1
WIDPDNTDTE

SEQ ID NO: 77 - protein, 13 aa, synthetic construct
  REGION 1..13: note = amino acid sequence of VH CDR3
NAAYGSSPYPMDY

SEQ ID NO: 78 - protein, 118 aa, synthetic construct
  REGION 1..118: note = VH chain region of the 9E4 antibody
EVQLRQSGPELVKPGASVKISCKASGYSFTDYYMYWVKQSRVRSLAWIGRINPYTGATGYDQNFKDKASLIVDKSSSTAYMELRSLTSEDSAVYYCARGRNRYDGWFAYWGQGTLVTV

SEQ ID NO: 79 - protein, 107 aa, synthetic construct
  REGION 1..107: note = VL chain region of the 9E4 antibody
EIQMTQTTSSLSASLGDRVTISCRASQDISNYLNWYQQKPDGTVKLLIYYTSRLHSGVPSRFSGSGSGTDYSLTISNLDQEDIATYFCQQGNALPPTFGGGTNLEIK

SEQ ID NO: 80 - protein, 115 aa, synthetic construct
  REGION 1..115: note = VH chain region of the 1B4 antibody
QIQLQQSGPELVKPGASVKISCKASGYTFTDYYIHWVKQRPGQGLEWIGWIYPGSGNTKYNERFKGKATLTVATSSSTAYMQLSSLTSEDTAVYFCARREEDYFDYWGQGTLVTV

SEQ ID NO: 81 - protein, 113 aa, synthetic construct
  REGION 1..113: note = VL chain region of the 1B4 antibody
DIVMSQSPSSLAVSVGEKVTMSCKSSQSLLYSSNQKNYLTWYQQKPGQSPKLLIYWASTRESGVPDRFTGSGSGTDFTLTISSVKAEDLAVYYCQQYYSYPLTFGAGTKLEIK

SEQ ID NO: 82 - DNA, 19 bp, synthetic construct
  misc_feature 1..19: note = Chemically synthesized oligonucleotide primer
  source 1..19: mol_type = other DNA
cactgcaggtrtccactcc

SEQ ID NO: 83 - DNA, 19 bp, synthetic construct
  misc_feature 1..19: note = Chemically synthesized oligonucleotide primer
  source 1..19: mol_type = other DNA
catagcaggtgtccactcc

SEQ ID NO: 84 - DNA, 19 bp, synthetic construct
  misc_feature 1..19: note = Chemically synthesized oligonucleotide primer
  source 1..19: mol_type = other DNA
crctacaggtgtccactcc

SEQ ID NO: 85 - DNA, 18 bp, synthetic construct
  misc_feature 1..18: note = Chemically synthesized oligonucleotide primer
  source 1..18: mol_type = other DNA
gcyacagmtgtccactcc

SEQ ID NO: 86 - DNA, 19 bp, synthetic construct
  misc_feature 1..19: note = Chemically synthesized oligonucleotide primer
  source 1..19: mol_type = other DNA
cactgcaggtgtccwmtcc

SEQ ID NO: 87 - DNA, 19 bp, synthetic construct
  misc_feature 1..19: note = Chemically synthesized oligonucleotide primer
  source 1..19: mol_type = other DNA
crctrcaggtgtkcactcc

SEQ ID NO: 88 - DNA, 18 bp, synthetic construct
  misc_feature 1..18: note = Chemically synthesized oligonucleotide primer
  source 1..18: mol_type = other DNA
gctawmggtgtccactcc

SEQ ID NO: 89 - DNA, 17 bp, synthetic construct
  misc_feature 1..17: note = Chemically synthesized oligonucleotide primer
  source 1..17: mol_type = other DNA
cctcaggtgtccactcc

SEQ ID NO: 90 - DNA, 18 bp, synthetic construct
  misc_feature 1..18: note = Chemically synthesized oligonucleotide primer
  source 1..18: mol_type = other DNA
gctacaggtgctcactcc

SEQ ID NO: 91 - DNA, 19 bp, synthetic construct
  misc_feature 1..19: note = Chemically synthesized oligonucleotide primer
  source 1..19: mol_type = other DNA
cactgcaggtgtcctctct

SEQ ID NO: 92 - DNA, 19 bp, synthetic construct
  misc_feature 1..19: note = Chemically synthesized oligonucleotide primer
  source 1..19: mol_type = other DNA
caytgcaggtgtccaytgc

SEQ ID NO: 93 - DNA, 18 bp, synthetic construct
  misc_feature 1..18: note = Chemically synthesized oligonucleotide primer
  source 1..18: mol_type = other DNA
gctammggtgtccacttc

SEQ ID NO: 94 - DNA, 21 bp, synthetic construct
  misc_feature 1..21: note = Chemically synthesized oligonucleotide primer
  source 1..21: mol_type = other DNA
ctcctgtcaktaactkcaggt

SEQ ID NO: 95 - DNA, 19 bp, synthetic construct
  misc_feature 1..19: note = Chemically synthesized oligonucleotide primer
  source 1..19: mol_type = other DNA
caactgcaggtgtctctct

SEQ ID NO: 96 - DNA, 19 bp, synthetic construct
  misc_feature 1..19: note = Chemically synthesized oligonucleotide primer
  source 1..19: mol_type = other DNA
crctrcaggygtccactct

SEQ ID NO: 97 - DNA, 18 bp, synthetic construct
  misc_feature 1..18: note = Chemically synthesized oligonucleotide primer
  source 1..18: mol_type = other DNA
ccaagctgtatcctttcc

SEQ ID NO: 98 - DNA, 18 bp, synthetic construct
  misc_feature 1..18: note = Chemically synthesized oligonucleotide primer
  source 1..18: mol_type = other DNA
ccaagctgtgtcctrtcc

SEQ ID NO: 99 - DNA, 19 bp, synthetic construct
  misc_feature 1..19: note = Chemically synthesized oligonucleotide primer
  source 1..19: mol_type = other DNA
cttgacagycvttcckggt

SEQ ID NO: 100 - DNA, 19 bp, synthetic construct
  misc_feature 1..19: note = Chemically synthesized oligonucleotide primer
  source 1..19: mol_type = other DNA
cttcacagcctttcctggt

SEQ ID NO: 101 - DNA, 19 bp, synthetic construct
  misc_feature 1..19: note = Chemically synthesized oligonucleotide primer
  source 1..19: mol_type = other DNA
cttaaaaggggtccagtgt

SEQ ID NO: 102 - DNA, 22 bp, synthetic construct
  misc_feature 1..22: note = Chemically synthesized oligonucleotide primer
  source 1..22: mol_type = other DNA
caytttaaaargtgtcmagtgt

SEQ ID NO: 103 - DNA, 20 bp, synthetic construct
  misc_feature 1..20: note = Chemically synthesized oligonucleotide primer
  source 1..20: mol_type = other DNA
gttttaaaaggtgtcctgtg

SEQ ID NO: 104 - DNA, 20 bp, synthetic construct
  misc_feature 1..20: note = Chemically synthesized oligonucleotide primer
  source 1..20: mol_type = other DNA
ctyttaaaaggkgtccagwg

SEQ ID NO: 105 - DNA, 21 bp, synthetic construct
  misc_feature 1..21: note = Chemically synthesized oligonucleotide primer
  source 1..21: mol_type = other DNA
cytttamatggtatccagtgt

SEQ ID NO: 106 - DNA, 21 bp, synthetic construct
  misc_feature 1..21: note = Chemically synthesized oligonucleotide primer
  source 1..21: mol_type = other DNA
cttttacatggtttcaagtgt

SEQ ID NO: 107 - DNA, 17 bp, synthetic construct
  misc_feature 1..17: note = Chemically synthesized oligonucleotide primer
  source 1..17: mol_type = other DNA
gtccctgcatatgtcyt

SEQ ID NO: 108 - DNA, 18 bp, synthetic construct
  misc_feature 1..18: note = Chemically synthesized oligonucleotide primer
  source 1..18: mol_type = other DNA
gatggcagcwgcycaaag

SEQ ID NO: 109 - DNA, 19 bp, synthetic construct
  misc_feature 1..19: note = Chemically synthesized oligonucleotide primer
  source 1..19: mol_type = other DNA
ctatcaaggtgtgcattgt

SEQ ID NO: 110 - DNA, 21 bp, synthetic construct
  misc_feature 1..21: note = Chemically synthesized oligonucleotide primer
  source 1..21: mol_type = other DNA
cttttaaaagwtgtccagkgt

SEQ ID NO: 111 - DNA, 20 bp, synthetic construct
  misc_feature 1..20: note = Chemically synthesized oligonucleotide primer
  source 1..20: mol_type = other DNA
gtgacagtccttcctggtag

SEQ ID NO: 112 - DNA, 19 bp, synthetic construct
  misc_feature 1..19: note = Chemically synthesized oligonucleotide primer
  source 1..19: mol_type = other DNA
cttcctgatggcagtggtt

SEQ ID NO: 113 - DNA, 18 bp, synthetic construct
  misc_feature 1..18: note = Chemically synthesized oligonucleotide primer
  source 1..18: mol_type = other DNA
gctacaggtatccaatcc

SEQ ID NO: 114 - DNA, 39 bp, synthetic construct
  misc_feature 1..39: note = Chemically synthesized oligonucleotide primer
  source 1..39: mol_type = other DNA
gcgtctagaayctccacacacaggrrccagtggatagac

SEQ ID NO: 115 - DNA, 19 bp, synthetic construct
  misc_feature 1..19: note = Chemically synthesized oligonucleotide primer
  source 1..19: mol_type = other DNA
ctgwtgttctggattcctg

SEQ ID NO: 116 - DNA, 18 bp, synthetic construct
  misc_feature 1..18: note = Chemically synthesized oligonucleotide primer
  source 1..18: mol_type = other DNA
ggtcagacagtcagcagt

SEQ ID NO: 117 - DNA, 18 bp, synthetic construct
  misc_feature 1..18: note = Chemically synthesized oligonucleotide primer
  source 1..18: mol_type = other DNA
gtgctctggattcgggaa

SEQ ID NO: 118 - DNA, 20 bp, synthetic construct
  misc_feature 1..20: note = Chemically synthesized oligonucleotide primer
  source 1..20: mol_type = other DNA
cagcttcytgctaatcagtg

SEQ ID NO: 119 - DNA, 18 bp, synthetic construct
  misc_feature 1..18: note = Chemically synthesized oligonucleotide primer
  source 1..18: mol_type = other DNA
ctaatcagtgcttcagga

SEQ ID NO: 120 - DNA, 20 bp, synthetic construct
  misc_feature 1..20: note = Chemically synthesized oligonucleotide primer
  source 1..20: mol_type = other DNA
gtgggtatctggtrcstgtg

SEQ ID NO: 121 - DNA, 23 bp, synthetic construct
  misc_feature 1..23: note = Chemically synthesized oligonucleotide primer
  source 1..23: mol_type = other DNA
ggaaatttaaaagtacctgtggg

SEQ ID NO: 122 - DNA, 20 bp, synthetic construct
  misc_feature 1..20: note = Chemically synthesized oligonucleotide primer
  source 1..20: mol_type = other DNA
ggtttcmaggtrccagatgt

SEQ ID NO: 123 - DNA, 18 bp, synthetic construct
  misc_feature 1..18: note = Chemically synthesized oligonucleotide primer
  source 1..18: mol_type = other DNA
ctctggttyccaggtatc

SEQ ID NO: 124 - DNA, 22 bp, synthetic construct
  misc_feature 1..22: note = Chemically synthesized oligonucleotide primer
  source 1..22: mol_type = other DNA
ctgttttcaaggtrccagatgt

SEQ ID NO: 125 - DNA, 18 bp, synthetic construct
  misc_feature 1..18: note = Chemically synthesized oligonucleotide primer
  source 1..18: mol_type = other DNA
gttgtaatgtccagagga

SEQ ID NO: 126 - DNA, 18 bp, synthetic construct
  misc_feature 1..18: note = Chemically synthesized oligonucleotide primer
  source 1..18: mol_type = other DNA
cttacaggtgccagatgt

SEQ ID NO: 127 - DNA, 22 bp, synthetic construct
  misc_feature 1..22: note = Chemically synthesized oligonucleotide primer
  source 1..22: mol_type = other DNA
ctcaattgtagrtgccagatgt

SEQ ID NO: 128 - DNA, 19 bp, synthetic construct
  misc_feature 1..19: note = Chemically synthesized oligonucleotide primer
  source 1..19: mol_type = other DNA
cacagtaggtgtcagatgt

SEQ ID NO: 129 - DNA, 18 bp, synthetic construct
  misc_feature 1..18: note = Chemically synthesized oligonucleotide primer
  source 1..18: mol_type = other DNA
gtcgtagttgtcagatgt

SEQ ID NO: 130 - DNA, 18 bp, synthetic construct
  misc_feature 1..18: note = Chemically synthesized oligonucleotide primer
  source 1..18: mol_type = other DNA
cctccttcttggccaaga

SEQ ID NO: 131 - DNA, 19 bp, synthetic construct
  misc_feature 1..19: note = Chemically synthesized oligonucleotide primer
  source 1..19: mol_type = other DNA
cttatatggagctgatggg

SEQ ID NO: 132 - DNA, 18 bp, synthetic construct
  misc_feature 1..18: note = Chemically synthesized oligonucleotide primer
  source 1..18: mol_type = other DNA
gtgtctggtgctcatggg

SEQ ID NO: 133 - DNA, 20 bp, synthetic construct
  misc_feature 1..20: note = Chemically synthesized oligonucleotide primer
  source 1..20: mol_type = other DNA
ctstggttgtctggtgttga

SEQ ID NO: 134 - DNA, 18 bp, synthetic construct
  misc_feature 1..18: note = Chemically synthesized oligonucleotide primer
  source 1..18: mol_type = other DNA
gtctctgattctagggca

SEQ ID NO: 135 - DNA, 16 bp, synthetic construct
  misc_feature 1..16: note = Chemically synthesized oligonucleotide primer
  source 1..16: mol_type = other DNA
ctkckctgggttccag

SEQ ID NO: 136 - DNA, 15 bp, synthetic construct
  misc_feature 1..15: note = Chemically synthesized oligonucleotide primer
  source 1..15: mol_type = other DNA
gcaggtgttgacgga

SEQ ID NO: 137 - DNA, 16 bp, synthetic construct
  misc_feature 1..16: note = Chemically synthesized oligonucleotide primer
  source 1..16: mol_type = other DNA
caggtgcctcgtgcac

SEQ ID NO: 138 - DNA, 16 bp, synthetic construct
  misc_feature 1..16: note = Chemically synthesized oligonucleotide primer
  source 1..16: mol_type = other DNA
ctctggtgcctgtgca

SEQ ID NO: 139 - DNA, 19 bp, synthetic construct
  misc_feature 1..19: note = Chemically synthesized oligonucleotide primer
  source 1..19: mol_type = other DNA
ctggaytycagcctccaga

SEQ ID NO: 140 - DNA, 19 bp, synthetic construct
  misc_feature 1..19: note = Chemically synthesized oligonucleotide primer
  source 1..19: mol_type = other DNA
gwtctctrgagtcagtggg

SEQ ID NO: 141 - DNA, 19 bp, synthetic construct
  misc_feature 1..19: note = Chemically synthesized oligonucleotide primer
  source 1..19: mol_type = other DNA
ctggatccctggakcyact

SEQ ID NO: 142 - DNA, 19 bp, synthetic construct
  misc_feature 1..19: note = Chemically synthesized oligonucleotide primer
  source 1..19: mol_type = other DNA
gttctgctttttaggtgtg

SEQ ID NO: 143 - DNA, 19 bp, synthetic construct
  misc_feature 1..19: note = Chemically synthesized oligonucleotide primer
  source 1..19: mol_type = other DNA
gatcccaggcatgatatgt

SEQ ID NO: 144 - DNA, 18 bp, synthetic construct
  misc_feature 1..18: note = Chemically synthesized oligonucleotide primer
  source 1..18: mol_type = other DNA
cttcatggtgctcagtgt

SEQ ID NO: 145 - DNA, 20 bp, synthetic construct
  misc_feature 1..20: note = Chemically synthesized oligonucleotide primer
  source 1..20: mol_type = other DNA
ccatatcaggtgcccagtgt

SEQ ID NO: 146 - DNA, 29 bp, synthetic construct
  misc_feature 1..29: note = Chemically synthesized oligonucleotide primer
  source 1..29: mol_type = other DNA
gcgtctagaactggatggtgggaagatgg

SEQ ID NO: 147 - protein, 305 aa, Homo sapiens
QLLFNKTKSVEFTFCNDTVVIPCFVTNMEAQNTTEVYVKWKFKGRDIYTFDGALNKSTVPTDFSSAKIEVSQLLKGDASLKMDKSDAVSHTGNYTCEVTELTREGETIIELKYRVVSWFSPNENILIVIFPIFAILLFWGQFGIKTLKYRSGGMDEKTIALLVAGLVITVIVIVGAILFVPGEYSLKNATGLGLIVTSTGILILLHYYVFSTAIGLTSFVIAILVIQVIAYILAVVGLSLCIAACIPMHGPLLISGLSILALAQLLGLVYMKFVASNQKTIQPPRKAVEEPLNAFKESKGMMNDE